European Patent Specification EP 3 883 600 B1, published March 12, 2025. Title: Bi-Specific Conjugates. Applicant: QUINE Medical AB. The sequence listing filed with the application follows.

SEQUENCE LISTING (155 sequences)

SEQ ID NO: 1 - protein, 8 aa, Gallus gallus
SIINFEKL

SEQ ID NO: 2 - protein, 9 aa, Mus musculus
EGSRNQDWL

SEQ ID NO: 3 - protein, 37 aa, Artificial Sequence
  UU-05 Peptide
FIGITELKKLESKINKVFLEQLESIINFEKLAAAAAK

SEQ ID NO: 4 - protein, 19 aa, Artificial Sequence
  UU-10 Peptide
LEQLESIINFEKLAAAAAK

SEQ ID NO: 5 - protein, 38 aa, Artificial Sequence
  UU-30 Peptide
FIGITELKKLESKINKVFAVGALKVPRNQDWLGVPRQL

SEQ ID NO: 6 - protein, 18 aa, Clostridium tetani
FIGITELKKLESKINKVF

SEQ ID NO: 7 - protein, 13 aa, Gallus gallus
LEQLESIINFEKL

SEQ ID NO: 8 - protein, 6 aa, Artificial Sequence
  UU-05 C-terminal sequence
AAAAAK

SEQ ID NO: 9 - protein, 20 aa, Artificial Sequence
  Human/murine gp100 fusion fragment
AVGALKVPRNQDWLGVPRQL

SEQ ID NO: 10 - protein, 22 aa, Clostridium tetani
GILFLQWVRDIIDDFTNESSQK

SEQ ID NO: 11 - protein, 21 aa, Clostridium tetani
DSDKDRFLQTMVKLFNRIKNN

SEQ ID NO: 12 - protein, 25 aa, Clostridium tetani
IDIKNDLYEKTLNDYKAIANKLSQV

SEQ ID NO: 13 - protein, 21 aa, Clostridium tetani
QDPALLLMHELIHVLHGLYGM

SEQ ID NO: 14 - protein, 24 aa, Clostridium tetani
DGILFLQWVRDIIDDFTNESSQKR

SEQ ID NO: 15 - protein, 326 aa, Artificial Sequence
  Human IgG2 C127S constant region
ASTKGPSVFPLAPSSRSTSESTAALGCLVKDYFPEPVTVSWNSGALTSGVHTFPAVLQSSGLYSLSSVVTVPSSNFGTQTYTCNVDHKPSNTKVDKTVERKCCVECPPCPAPPVAGPSVFLFPPKPKDTLMISRTPEVTCVVVDVSHEDPEVQFNWYVDGVEVHNAKTKPREEQFNSTFRVVSVLTVVHQDWLNGKEYKCKVSNKGLPAPIEKTISKTKGQPREPQVYTLPPSREEMTKNQVSLTCLVKGFYPSDIAVEWESNGQPENNYKTTPPMLDSDGSFFLYSKLTVDKSRWQQGNVFSCSVMHEALHNHYTQKSLSLSPGK

SEQ ID NO: 16 - protein, 1315 aa, Clostridium tetani
MPITINNFRYSDPVNNDTIIMMEPPYCKGLDIYYKAFKITDRIWIVPERYEFGTKPEDFNPPSSLIEGASEYYDPNYLRTDSDKDRFLQTMVKLFNRIKNNVAGEALLDKIINAIPYLGNSYSLLDKFDTNSNSVSFNLLEQDPSGATTKSAMLTNLIIFGPGPVLNKNEVRGIVLRVDNKNYFPCRDGFGSIMQMAFCPEYVPTFDNVIENITSLTIGKSKYFQDPALLLMHELIHVLHGLYGMQVSSHEIIPSKQEIYMQHTYPISAEELFTFGGQDANLISIDIKNDLYEKTLNDYKAIANKLSQVTSCNDPNIDIDSYKQIYQQKYQFDKDSNGQYIVNEDKFQILYNSIMYGFTEIELGKKFNIKTRLSYFSMNHDPVKIPNLLDDTIYNDTEGFNIESKDLKSEYKGQNMRVNTNAFRNVDGSGLVSKLIGLCKKIIPPTNIRENLYNRTASLTDLGGELCIKIKNEDLTFIAEKNSFSEEPFQDEIVSYNTKNKPLNFNYSLDKIIVDYNLQSKITLPNDRTTPVTKGIPYAPEYKSNAASTIEIHNIDDNTIYQYLYAQKSPTTLQRITMTNSVDDALINSTKIYSYFPSVISKVNQGAQGILFLQWVRDIIDDFTNESSQKTTIDKISDVSTIVPYIGPALNIVKQGYEGNFIGALETTGVVLLLEYIPEITLPVIAALSIAESSTQKEKIIKTIDNFLEKRYEKWIEVYKLVKAKWLGTVNTQFQKRSYQMYRSLEYQVDAIKKIIDYEYKIYSGPDKEQIADEINNLKNKLEEKANKAMININIFMRESSRSFLVNQMINEAKKQLLEFDTQSKNILMQYIKANSKFIGITELKKLESKINKVFSTPIPFSYSKNLDCWVDNEEDIDVILKKSTILNLDINNDIISDISGFNSSVITYPDAQLVPGINGKAIHLVNNESSEVIVHKAMDIEYNDMFNNFTVSFWLRVPKVSASHLEQYGTNEYSIISSMKKHSLSIGSGWSVSLKGNNLIWTLKDSAGEVRQITFRDLPDKFNAYLANKWVFITITNDRLSSANLYINGVLMGSAEITGLGAIREDNNITLKLDRCNNNNQYVSIDKFRIFCKALNPKEIEKLYTSYLSITFLRDFWGNPLRYDTEYYLIPVASSSKDVQLKNITDYMYLTNAPSYTNGKLNIYYRRLYNGLKFIIKRYTPNNEIDSFVKSGDFIKLYVSYNNNEHIVGYPKDGNAFNNLDRILRVGYNAPGIPLYKKMEAVKLRDLKTYSVQLKLYDDKNASLGLVGTHNGQIGNDPNRDILIASNWYFNHLKDKILGCDWYFVPTDEGWTND

SEQ ID NO: 17 - protein, 8 aa, Artificial Sequence
  ABS-1150 VHCDR1
GFTFSSYA

SEQ ID NO: 18 - protein, 8 aa, Artificial Sequence
  ABS-1150 VHCDR2
IGGSSSYT

SEQ ID NO: 19 - protein, 10 aa, Artificial Sequence
  ABS-1150 VHCDR3
ARYYSYHMDY

SEQ ID NO: 20 - protein, 6 aa, Artificial Sequence
  ABS-1150 VLCDR1
QSISSY

SEQ ID NO: 21 - protein, 3 aa, Artificial Sequence
  ABS-1150 VLCDR2
AAS

SEQ ID NO: 22 - protein, 9 aa, Artificial Sequence
  ABS-1150 VLCDR3
QQYGSAPPT

SEQ ID NO: 23 - protein, 117 aa, Artificial Sequence
  ABS-1150 Heavy Chain Variable Domain
EVQLLESGGGLVQPGGSLRLSCAASGFTFSSYAMSWVRQAPGKGLEWVSGIGGSSSYTSYADSVKGRFTISRDNSKNTLYLQMNSLRAEDTAVYYCARYYSYHMDYWGQGTLVTVSS

SEQ ID NO: 24 - protein, 107 aa, Artificial Sequence
  ABS-1150 Light Chain Variable Domain
DIQMTQSPSSLSASVGDHVTITCRASQSISSYLNWYQQKPGKAPKLLIYAASSLQSGVPSRFSGSGSGTDFTLTISSLQPEDFATYYCQQYGSAPPTFGQGTKLEIK

SEQ ID NO: 25 - DNA, 351 bp, Artificial Sequence
  ABS-1150 Heavy Chain Variable Domain
gaggtgcagctgttggagagcgggggaggcttggtacagcctggggggtccctgcgcctctcctgtgcagccagcggattcacctttagcagctatgccatgagctgggtccgccaggctccagggaaggggctggagtgggtctcaggtattggtggttcttcttcttacacatcttatgcagactccgtgaagggccggttcaccatctcccgtgacaattccaagaacacgctgtatctgcaaatgaacagcctgcgtgccgaggacacggctgtatattattgtgcgcgctactactcttaccatatggactattggggccagggaaccctggtcaccgtctcctca

SEQ ID NO: 26 - DNA, 321 bp, Artificial Sequence
  ABS-1150 Light Chain Variable Domain
gacatccagatgacccagtctccatcctccctgagcgcatctgtaggagaccacgtcaccatcacttgccgggcaagtcagagcattagcagctatttaaattggtatcagcagaaaccagggaaagcccctaagctcctgatctatgctgcatccagtttgcaaagtggggtcccatcacgtttcagtggcagtggaagcgggacagatttcactctcaccatcagcagtctgcaacctgaagattttgcaacttattactgtcaacagtacggttctgctccgcccacttttggccaggggaccaagctggagatcaaa

SEQ ID NO: 27 - protein, 126 aa, Artificial Sequence
  CP-870,893 Heavy Chain Variable Domain
QVQLVQSGAEVKKPGASVKVSCKASGYTFTGYYMHWVRQAPGQGLEWMGWINPDSGGTNYAQKFQGRVTMTRDTSISTAYMELNRLRSDDTAVYYCARDQPLGYCTNGVCSYFDYWGQGTLVTVSS

SEQ ID NO: 28 - protein, 107 aa, Artificial Sequence
  CP-870,893 Light Chain Variable Domain
DIQMTQSPSSVSASVGDRVTITCRASQGIYSWLAWYQQKPGKAPNLLIYTASTLQSGVPSRFSGSGSGTDFTLTISSLQPEDFATYYCQQANIFPLTFGGGTKVEIK

SEQ ID NO: 29 - DNA, 378 bp, Artificial Sequence
  CP-870,893 Heavy Chain Variable Domain
caggtgcagctggtgcagtctggagctgaggtgaagaaaccaggagcttctgtgaaggtgagttgcaaagcctcaggctacaccttcacagggtactatatgcactgggtgcggcaggctcctggacagggcctggaatggatgggctggatcaaccctgactctggcgggaccaattacgcccagaagtttcaggggagggtgactatgacccgcgataccagcatttccacagcttatatggagctgaaccggctgagaagcgacgatactgccgtgtactattgtgctagggaccagcccctgggatattgcaccaatggcgtgtgcagctacttcgattattgggggcagggaacactggtgaccgtgagctca

SEQ ID NO: 30 - DNA, 321 bp, Artificial Sequence
  CP-870,893 Light Chain Variable Domain
gacatccagatgacccagtctcctagctccgtgtcagcctctgtgggcgatagagtgaccatcacatgcagagcctctcaggggatctactcctggctggcttggtatcagcagaagcccggcaaagcccctaacctgctgatctacacagcttcaactctgcagtctggagtgccctcccggttctccggctctgggagtggaactgactttactctgaccatttctagtctgcagccagaggatttcgccacctactattgtcagcaggctaatatcttccccctgacctttggcgggggaacaaaggtggaaattaaa

SEQ ID NO: 31 - protein, 8 aa, Artificial Sequence
  ADC-1013 VHCDR1 (IMGT)
GFTFSTYG

SEQ ID NO: 32 - protein, 8 aa, Artificial Sequence
  ADC-1013 VHCDR2 (IMGT)
ISGGSSYI

SEQ ID NO: 33 - protein, 12 aa, Artificial Sequence
  ADC-1013 VHCDR3 (IMGT)
ARILRGGSGMDL

SEQ ID NO: 34 - protein, 9 aa, Artificial Sequence
  ADC-1013 VLCDR1 (IMGT)
SSNIGAGYN

SEQ ID NO: 35 - protein, 4 aa, Artificial Sequence
  ADC-1013 VLCDR2 (IMGT)
GNIN

SEQ ID NO: 36 - protein, 11 aa, Artificial Sequence
  ADC-1013 VLCDR3 (IMGT)
AAWDKSISGLV

SEQ ID NO: 37 - protein, 119 aa, Artificial Sequence
  ADC-1013 Heavy Chain Variable Domain
EVQLLESGGGLVQPGGSLRLSCAASGFTFSTYGMHVWRQAPGKGLEWLSYISGGSSYIFYADSVRGRFTISRDNSENALYLQMNSLRAEDTAVYYCARILRGGSGMDLWGQGTLVTVSS

SEQ ID NO: 38 - protein, 112 aa, Artificial Sequence
  ADC-1013 Light Chain Variable Domain
QSVLTQPPSASGTPGQRVTISCTGSSSNIGAGYNVYWYQQLPGTAPKLLIYGNINRPSGVPDRFSGSKSGTSASLAISGLRSEDEADYYCAAWDKSISGLVFGGGTKLTVLG

SEQ ID NO: 39 - DNA, 357 bp, Artificial Sequence
  ADC-1013 Heavy Chain Variable Domain
gaggtgcagctgttggagtctgggggaggcttggtacagcctggggggtccctgagactctcctgtgcagcctctggattcaccttcagtacttatggcatgcactgggtccgccaggctccagggaaggggctggagtggctttcatatattagtggtggtagtagttacattttctacgcagactcagtgaggggccgattcaccatctccagagacaactccgagaacgcgctgtatctgcaaatgaacagcctgagagccgaggacacggccgtgtattactgtgcgagaatattaagaggcgggagcggtatggacctctggggccaaggtacactggtcaccgtgagctca

SEQ ID NO: 40 - DNA, 336 bp, Artificial Sequence
  ADC-1013 Light Chain Variable Domain
cagtctgtgctgactcagccaccctcagcgtctgggacccccgggcagagggtcaccatctcttgcactgggagcagctccaacatcggggcgggttacaatgtatactggtatcagcagctcccaggaacggcccccaaactcctcatctatggtaacatcaatcggccctcaggggtccctgaccgattctctggctccaagtctggcacctcagcctccctggccatcagtgggctccggtccgaggatgaggctgattattactgtgcagcatgggataagagcatttctggtctggttttcggcggaggaaccaagctgacggtcctaggt

SEQ ID NO: 41 - protein, 330 aa, Homo sapiens [sequence omitted]

SEQ ID NO: 42 - protein, 326 aa, Homo sapiens
ASTKGPSVFPLAPCSRSTSESTAALGCLVKDYFPEPVTVSWNSGALTSGVHTFPAVLQSSGLYSLSSVVTVPSSNFGTQTYTCNVDHKPSNTKVDKTVERKCCVECPPCPAPPVAGPSVFLFPPKPKDTLMISRTPEVTCVVVDVSHEDPEVQFNWYVDGVEVHNAKTKPREEQFNSTFRVVSVLTVVHQDWLNGKEYKCKVSNKGLPAPIEKTISKTKGQPREPQVYTLPPSREEMTKNQVSLTCLVKGFYPSDISVEWESNGQPENNYKTTPPMLDSDGSFFLYSKLTVDKSRWQQGNVFSCSVMHEALHNHYTQKSLSLSPGK

SEQ ID NO: 43 - protein, 377 aa, Homo sapiens
ASTKGPSVFPLAPCSRSTSGGTAALGCLVKDYFPEPVTVSWNSGALTSGVHTFPAVLQSSGLYSLSSVVTVPSSSLGTQTYTCNVNHKPSNTKVDKRVELKTPLGDTTHTCPRCPEPKSCDTPPPCPRCPEPKSCDTPPPCPRCPEPKSCDTPPPCPRCPAPELLGGPSVFLFPPKPKDTLMISRTPEVTCVVVDVSHEDPEVQFKWYVDGVEVHNAKTKPREEQYNSTFRVVSVLTVLHQDWLNGKEYKCKVSNKALPAPIEKTISKTKGQPREPQVYTLPPSREEMTKNQVSLTCLVKGFYPSDIAVEWESSGQPENNYNTTPPMLDSDGSFFLYSKLTVDKSRWQQGNIFSCSVMHEALHNRFTQKSLSLSPGK

SEQ ID NO: 44 - protein, 327 aa, Homo sapiens
ASTKGPSVFPLAPCSRSTSESTAALGCLVKDYFPEPVTVSWNSGALTSGVHTFPAVLQSSGLYSLSSVVTVPSSSLGTKTYTCNVDHKPSNTKVDKRVESKYGPPCPSCPAPEFLGGPSVFLFPPKPKDTLMISRTPEVTCVVVDVSQEDPEVQFNWYVDGVEVHNAKTKPREEQFNSTYRVVSVLTVLHQDWLNGKEYKCKVSNKGLPSSIEKTISKAKGQPREPQVYTLPPSQEEMTKNQVSLTCLVKGFYPSDIAVEWESNGQPENNYKTTPPVLDSDGSFFLYSRLTVDKSRWQEGNVFSCSVMHEALHNHYTQKSLSLSLGK

SEQ ID NO: 45 - protein, 107 aa, Homo sapiens [sequence omitted]

SEQ ID NO: 46 - protein, 106 aa, Homo sapiens
GQPKANPTVTLFPPSSEELQANKATLVCLISDFYPGAVTVAWKADGSPVKAGVETTKPSKQSNNKYAASSYLSLTPEQWKSHRSYSCQVTHEGSTVEKTVAPTECS

SEQ ID NO: 47 - protein, 244 aa, Artificial Sequence
  14GIIICII scFv
QVQLQQPGAELVMPGASVNLSCKASGYTFTDYWMHWVKQRPGQGLEWIGEIDPSDNFSNLNQNFRGKATLTVDKSSRTAFLQLSSLTSEDSAVYYCAVEDYWGQGTTLTVSSGGGGSGGGGSGGGGSGGGGSDIVMTQATPSVLVTPGEAVSISCRASRSLLHSNGITYLYWFLQRPGQSPQVLIYRMSNLVSGVPDRFSGSGSGTAFTLRISRVEAEDVGVYYCMQHLEFPYTFGGGTKLEIK

SEQ ID NO: 48 - protein, 245 aa, Artificial Sequence
  IBIIICI-b scFv
EVRLLQSGAALVRPGASVKLSCTASGFNIKDFNIHWVKQRPEQGLEWIGRIDPENGDAEYVPKFQVRATMTTDTSSNTVYLHLSSLTSGDTAVYYCTTGSYDLDVEYWGQGTTLTVSSGGGGSGGGGSGGGGSGGGGSELQMTQSPSSLSASLGDTVTITCHASQNINVWLSWYQQRPGNIPKLLIYKASTLHTGVPSRFRGSGSGTGFTLTISSLQPEDIATYYCQQGQSYPLTFGAGTKLELK

SEQ ID NO: 49 - protein, 10 aa, Artificial Sequence
  GGGGS2 Linker
GGGGSGGGGS

SEQ ID NO: 50 - protein, 277 aa, Homo sapiens
MVRLPLQCVLWGCLLTAVHPEPPTACREKQYLINSQCCSLCQPGQKLVSDCTEFTETECLPCGESEFLDTWNRETHCHQHKYCDPNLGLRVQQKGTSETDTICTCEEGWHCTSEACESCVLHRSCSPGFGVKQIATGVSDTICEPCPVGFFSNVSSAFEKCHPWTSCETKDLVVQQAGTNKTDVVCGPQDRLRALVVIPIIFGILFAILLVLVFIKKVAKKPTNKAPHPKQEPQEINFPDDLPGSNTAAPVQETLHGCQPVTQEDGKESRISVQERQ

SEQ ID NO: 51 - protein, 5 aa, Artificial Sequence
  GGGGS linker module
GGGGS

SEQ ID NO: 52 - protein, 122 aa, Artificial Sequence
  ChiLob 7/4 Heavy Chain Variable Domain
EVQLQQSGPDLVKPGASVKISCKTSGYTFTEYIMHWVKQSHGKSLEWIGGIIPNNGGTSYNQKFKDKATMTVDKSSSTGYMELRSLTSEDSAVYYCTRREVYGRNYYALDYWGQGTLVTVSS

SEQ ID NO: 53 - protein, 107 aa, Artificial Sequence
  ChiLob 7/4 Light Chain Variable Domain
DIQMTQTTSSLSASLGDRVTITCSASQGINNYLNWYQQKPDGTVKLLIYYTSSLHSGVPSRFSGSGSGTDYSLTISNLEPEDIATYYCQQYSNLPYTFGGGTKLEIK

SEQ ID NO: 54 - protein, 114 aa, Artificial Sequence [sequence omitted]

SEQ ID NO: 55 - protein, 112 aa, Artificial Sequence [sequence omitted]

SEQ ID NO: 56 - protein, 120 aa, Artificial Sequence
  APX-005M Heavy Chain Variable Domain
QVQLVESGGGVVQPGRSLRLSCAASGFSFSSTYVCWVRQAPGKGLEWIACIYTGDGTNYSASWAKGRFTISKDSSKNTVYLQMNSLRAEDTAVYFCARPDITYGFAINFWGPGTLVTVSS

SEQ ID NO: 57 - protein, 108 aa, Artificial Sequence
  APX-005M Light Chain Variable Domain
DIQMTQSPSSLSASVGDRVTIKCQASQSISSRLAWYQQKPGKPPKLLIYRASTLASGVPSRFSGSGSGTDFTLTISSLQPEDVATYYCQCTGYGISWPIGGGTKVEIK

SEQ ID NO: 58 - protein, 9 aa, Artificial Sequence
  APX-005M VHCDR1 (IMGT)
GFSFSSTYV

SEQ ID NO: 59 - protein, 8 aa, Artificial Sequence
  APX-005M VHCDR2 (IMGT)
IYTGDGTN

SEQ ID NO: 60 - protein, 13 aa, Artificial Sequence
  APX-005M VHCDR3 (IMGT)
ARPDITYGFAINF

SEQ ID NO: 61 - protein, 6 aa, Artificial Sequence
  APX-005M VLCDR1 (IMGT)
QSISSR

SEQ ID NO: 62 - protein, 3 aa, Artificial Sequence
  APX-005M VLCDR2 (IMGT)
RAS

SEQ ID NO: 63 - protein, 7 aa, Artificial Sequence
  APX-005M VLCDR3 (IMGT)
QCTGYGI

SEQ ID NO: 64 - protein, 8 aa, Artificial Sequence
  CP-870,893 VHCDR1
GYTFTGYY

SEQ ID NO: 65 - protein, 8 aa, Artificial Sequence
  CP-870,893 VHCDR2
INPDSGGT

SEQ ID NO: 66 - protein, 19 aa, Artificial Sequence
  CP-870,893 VHCDR3
ARDQPLGYCTNGVCSYFDY

SEQ ID NO: 67 - protein, 6 aa, Artificial Sequence
  CP-870,893 VLCDR1
QGIYSW

SEQ ID NO: 68 - protein, 3 aa, Artificial Sequence
  CP-870,893 VLCDR2
TAS

SEQ ID NO: 69 - protein, 9 aa, Artificial Sequence
  CP-870,893 VLCDR3
QQANIFPLT

SEQ ID NO: 70 - protein, 248 aa, Artificial Sequence
  FITC-8 scFv
EVQLLESGGGLVQPGGSLRLSCAASGFTFSNYWMSWVRQAPGKGLEWVSGISGNGGYTYFADSVKDRFTISRDNSKNTLYLQMNSLRAEDTAVYYCAGGDGSGWSFWGQGTLVTVSSGGGGSGGGGSGGGGSGGGGSQSVLTQPPSASGTPGQRVTISCTGSSSNIGAGYDVHWYQQLPGTAPKLLIYGNNNRPSGVPDRFSGSKSGTSASLAISGLRSEDEADYYCAAWDDSLSGRVFGGGTKLTVL

SEQ ID NO: 71 - protein, 22 aa, Artificial Sequence
  Peptide UU-44
AGILARNLVPMVATVQGQNLKY

SEQ ID NO: 72 - protein, 9 aa, Human cytomegalovirus
NLVPMVATV

SEQ ID NO: 73 - protein, 37 aa, Clostridium tetani
DANLISIDIKNDLYEKTLNDYKAIANKLSQVTSCNDP

SEQ ID NO: 74 - protein, 37 aa, Clostridium tetani
TIGKSKYFQDPALLLMHELIHVLHGLYGMQVSSHEII

SEQ ID NO: 75 - protein, 15 aa, Clostridium tetani
DANLISIDIKNDLYE

SEQ ID NO: 76 - protein, 15 aa, Clostridium tetani
ANLISIDIKNDLYEK

SEQ ID NO: 77 - protein, 15 aa, Clostridium tetani
NLISIDIKNDLYEKT

SEQ ID NO: 78 - protein, 15 aa, Clostridium tetani
LISIDIKNDLYEKTL

SEQ ID NO: 79 - protein, 15 aa, Clostridium tetani
ISIDIKNDLYEKTLN

SEQ ID NO: 80 - protein, 15 aa, Clostridium tetani
SIDIKNDLYEKTLND

SEQ ID NO: 81 - protein, 15 aa, Clostridium tetani
IDIKNDLYEKTLNDY

SEQ ID NO: 82 - protein, 15 aa, Clostridium tetani
DIKNDLYEKTLNDYK

SEQ ID NO: 83 - protein, 15 aa, Clostridium tetani
IKNDLYEKTLNDYKA

SEQ ID NO: 84 - protein, 15 aa, Clostridium tetani
KNDLYEKTLNDYKAI

SEQ ID NO: 85 - protein, 15 aa, Clostridium tetani
NDLYEKTLNDYKAIA

SEQ ID NO: 86 - protein, 15 aa, Clostridium tetani
DLYEKTLNDYKAIAN

SEQ ID NO: 87 - protein, 15 aa, Clostridium tetani
LYEKTLNDYKAIANK

SEQ ID NO: 88 - protein, 15 aa, Clostridium tetani
YEKTLNDYKAIANKL

SEQ ID NO: 89 - protein, 15 aa, Clostridium tetani
EKTLNDYKAIANKLS

SEQ ID NO: 90 - protein, 15 aa, Clostridium tetani
KTLNDYKAIANKLSQ

SEQ ID NO: 91 - protein, 15 aa, Clostridium tetani
TLNDYKAIANKLSQV

SEQ ID NO: 92 - protein, 15 aa, Clostridium tetani
LNDYKAIANKLSQVT

SEQ ID NO: 93 - protein, 15 aa, Clostridium tetani
NDYKAIANKLSQVTS

SEQ ID NO: 94 - protein, 15 aa, Clostridium tetani
DYKAIANKLSQVTSC

SEQ ID NO: 95 - protein, 15 aa, Clostridium tetani
YKAIANKLSQVTSCN

SEQ ID NO: 96 - protein, 15 aa, Clostridium tetani
KAIANKLSQVTSCND

SEQ ID NO: 97 - protein, 15 aa, Clostridium tetani
AIANKLSQVTSCNDP

SEQ ID NO: 98 - protein, 15 aa, Clostridium tetani
TIGKSKYFQDPALLL

SEQ ID NO: 99 - protein, 15 aa, Clostridium tetani
IGKSKYFQDPALLLM

SEQ ID NO: 100 - protein, 15 aa, Clostridium tetani
GKSKYFQDPALLLMH

SEQ ID NO: 101 - protein, 15 aa, Clostridium tetani
KSKYFQDPALLLMHE

SEQ ID NO: 102 - protein, 15 aa, Clostridium tetani
SKYFQDPALLLMHEL

SEQ ID NO: 103 - protein, 15 aa, Clostridium tetani
KYFQDPALLLMHELI

SEQ ID NO: 104 - protein, 15 aa, Clostridium tetani
YFQDPALLLMHELIH

SEQ ID NO: 105 - protein, 15 aa, Clostridium tetani
FQDPALLLMHELIHV

SEQ ID NO: 106 - protein, 15 aa, Clostridium tetani
QDPALLLMHELIHVL

SEQ ID NO: 107 - protein, 15 aa, Clostridium tetani
DPALLLMHELIHVLH

SEQ ID NO: 108 - protein, 15 aa, Clostridium tetani
PALLLMHELIHVLHG

SEQ ID NO: 109 - protein, 15 aa, Clostridium tetani
ALLLMHELIHVLHGL

SEQ ID NO: 110 - protein, 15 aa, Clostridium tetani
LLLMHELIHVLHGLY

SEQ ID NO: 111 - protein, 15 aa, Clostridium tetani
LLMHELIHVLHGLYG

SEQ ID NO: 112 - protein, 15 aa, Clostridium tetani
LMHELIHVLHGLYGM

SEQ ID NO: 113 - protein, 15 aa, Clostridium tetani
MHELIHVLHGLYGMQ

SEQ ID NO: 114 - protein, 15 aa, Clostridium tetani
HELIHVLHGLYGMQV

SEQ ID NO: 115 - protein, 15 aa, Clostridium tetani
ELIHVLHGLYGMQVS

SEQ ID NO: 116 - protein, 15 aa, Clostridium tetani
LIHVLHGLYGMQVSS

SEQ ID NO: 117 - protein, 15 aa, Clostridium tetani
IHVLHGLYGMQVSSH

SEQ ID NO: 118 - protein, 15 aa, Clostridium tetani
HVLHGLYGMQVSSHE

SEQ ID NO: 119 - protein, 15 aa, Clostridium tetani
VLHGLYGMQVSSHEI

SEQ ID NO: 120 - protein, 15 aa, Clostridium tetani
LHGLYGMQVSSHEII

SEQ ID NO: 121 - protein, 11 aa, Clostridium tetani
NDYKAIANKLS

SEQ ID NO: 122 - protein, 13 aa, Clostridium tetani
LMHELIHVLHGLY

SEQ ID NO: 123 - protein, 15 aa, Clostridium tetani
LMHELIHVLHGLYGM

SEQ ID NO: 124 - protein, 9 aa, Clostridium tetani
LIHVLHGLY

SEQ ID NO: 125 - protein, 14 aa, Clostridium tetani
PALLLMHELIHVLH

SEQ ID NO: 126 - protein, 8 aa, Artificial Sequence
  14GIIICII-b scFv VHCDR1
GYTFTDYW

SEQ ID NO: 127 - protein, 8 aa, Artificial Sequence
  14GIIICII-b scFv VHCDR2
IDPSDNFS

SEQ ID NO: 128 - protein, 5 aa, Artificial Sequence
  14GIIICII-b scFv VHCDR3
AVEDY

SEQ ID NO: 129 - protein, 11 aa, Artificial Sequence
  14GIIICII-b scFv VLCDR1
RSLLHSNGITY

SEQ ID NO: 130 - protein, 3 aa, Artificial Sequence
  14GIIICII-b scFv VLCDR2
RMS

SEQ ID NO: 131 - protein, 9 aa, Artificial Sequence
  14GIIICII-b scFv VLCDR3
MQHLEFPYT

SEQ ID NO: 132 - protein, 8 aa, Artificial Sequence
  1BIIICI-b scFv VHCDR1
GFNIKDFN

SEQ ID NO: 133 - protein, 8 aa, Artificial Sequence
  1BIIICI-b VHCDR2
IDPENGDA

SEQ ID NO: 134 - protein, 11 aa, Artificial Sequence
  1BIIICI-b scFv VHCDR3
TTGSYDLDVEY

SEQ ID NO: 135 - protein, 6 aa, Artificial Sequence
  1BIIICI-b scFv VLCDR1
QNINVW

SEQ ID NO: 136 - protein, 3 aa, Artificial Sequence
  1BIIICI-b scFv VLCDR2
KAS

SEQ ID NO: 137 - protein, 9 aa, Artificial Sequence
  1BIIICI-b scFv VLCDR3
QQGQSYPLT

SEQ ID NO: 138 - protein, 10 aa, Artificial Sequence
  ADC-1013 VHCDR1 (Kabat)
GFTFSTYGMH

SEQ ID NO: 139 - protein, 26 aa, Artificial Sequence
  ADC-1013 VHCDR2 (Kabat)
GKGLEWLSYISGGSSYIFYADSVRGR

SEQ ID NO: 140 - protein, 13 aa, Artificial Sequence
  ADC-1013 VHCDR3 (Kabat)
CARILRGGSGMDL

SEQ ID NO: 141 - protein, 15 aa, Artificial Sequence
  ADC-1013 VLCDR1 (Kabat)
CTGSSSNIGAGYNVY

SEQ ID NO: 142 - protein, 7 aa, Artificial Sequence
  ADC-1013 VLCDR2 (Kabat)
GNINRPS

SEQ ID NO: 143 - protein, 12 aa, Artificial Sequence
  ADC-1013 VLCDR3 (Kabat)
CAAWDKSISGLV

SEQ ID NO: 144 - protein, 10 aa, Artificial Sequence
  APX-005M VHCDR1 (Kabat)
GFSFSSTYVC

SEQ ID NO: 145 - protein, 17 aa, Artificial Sequence
  APX-005M VHCDR2 (Kabat)
CIYTGDGTNYSASWAKG

SEQ ID NO: 146 - protein, 13 aa, Artificial Sequence
  APX-005M VHCDR3 (Kabat)
ARPDITYGFAINF

SEQ ID NO: 147 - protein, 11 aa, Artificial Sequence
  APX-005M VLCDR1 (Kabat)
QASQSISSRLA

SEQ ID NO: 148 - protein, 7 aa, Artificial Sequence
  APX-005M VLCDR2 (Kabat)
RASTLAS

SEQ ID NO: 149 - protein, 10 aa, Artificial Sequence
  APX-005M VLCDR3 (Kabat)
QCTGYGISWP

SEQ ID NO: 150 - protein, 240 aa, Artificial Sequence
  Y-SM083-p03-C06 scFv
EVQLLESGGGLVQPGGSLRLSCAASGFTFSSYAMSWVRQAPGKGLEWVSSISSSSGSTYYADSVKGRFTISRDNSKNTLYLQMNSLRAEDTAVYYCARHGRWGYYFDYWGQGTLVTVSSGGGGSGGGGSGGGGSDIQMTQSPSSLSASVGDRVTITCRASQSISSYLNWYQQKPGKAPKLLIYAASSLQSGVPSRFSGSGSGTDFTLTISSLQPEDFATYYCQQISGPFTFGQGTKLEIK

SEQ ID NO: 151 - protein, 243 aa, Artificial Sequence
  Y-SM083-p04-C04 scFv
EVQLLESGGGLVQPGGSLRLSCAASGFTFSSYAMSWVRQAPGKGLEWVSAISGSGGSTYYADSVKGRFTISRDNSKNTLYLQMNSLRAEDTAVYYCARTPPPSSSRSYLDYWGQGTLVTVSSGGGGSGGGGSGGGGSDIQMTQSPSSLSASVGDRVTITCRASQSISSYLNWYQQKPGKAPKLLIYAASSLQSGVPSRFSGSGSGTDFTLTISSLQPEDFATYYCQQYYPLFTFGQGTKLEIK

SEQ ID NO: 152 - protein, 239 aa, Artificial Sequence
  Y-SM083-p04-D04 scFv
EVQLLESGGGLVQPGGSLRLSCAASGFTFSGYYMYWVRQAPGKGLEWVSYIGYSGGGTGYADSVKGRFTISRDNSKNTLYLQMNSLRAEDTAVYYCARVPFGAFDYWGQGTLVTVSSGGGGSGGGGSGGGGSDIQMTQSPSSLSASVGDRVTITCRASQSISSYLNWYQQKPGKAPKLLIYAASSLQSGVPSRFSGSGSGTDFTLTISSLQPEDFATYYCQQYYGFPYTFGQGTKLEIK

SEQ ID NO: 153 - protein, 244 aa, Artificial Sequence
  Y-SM083-p04-F04 scFv
EVQLLESGGGLVQPGGSLRLSCAASGFTFSSYAMSWVRQAPGKGLEWVSAISGSGGSTYYADSVKGRFTISRDNSKNTLYLQMNSLRAEDTAVYYCARYPRPYSIFISIDYWGQGTLVTVSSGGGGSGGGGSGGGGSDIQMTQSPSSLSASVGDRVTITCRASQSISSYLNWYQQKPGKAPKLLIYAASSLQSGVPSRFSGSGSGTDFTLTISSLQPEDFATYYCQQTYGTPFTFGQGTKLEIK

SEQ ID NO: 154 - protein, 243 aa, Artificial Sequence
  Y-SM083-p04-G04 scFv
EVQLLESGGGLVQPGGSLRLSCAASGFTFSSYAMSWVRQAPGKGLEWVSAISGSGGSTYYADSVKGRFTISRDNSKNTLYLQMNSLRAEDTAVYYCARYSVPYSPYYSFDYWGQGTLVTVSSGGGGSGGGGSGGGGSDIQMTQSPSSLSASVGDRVTITCRASQSISSYLNWYQQKPGKAPKLLIYAASSLQSGVPSRFSGSGSGTDFTLTISSLQPEDFATYYCQQTYSPPTFGQGTKLEIK

SEQ ID NO: 155 - protein, 243 aa, Artificial Sequence
  Y-SM083-p04-H04 scFv
EVQLLESGGGLVQPGGSLRLSCAASGFTFSSYAMSWVRQAPGKGLEWVSAISGSGGSTYYADSVKGRFTISRDNSKNTLYLQMNSLRAEDTAVYYCARYTYGGFPFSSFDYWGQGTLVTVSSGGGGSGGGGSGGGGSDIQMTQSPSSLSASVGDRVTITCRASQSISSYLNWYQQKPGKAPKLLIYAASSLQSGVPSRFSGSGSGTDFTLTISSLQPEDFATYYCQQYRFLSTFGQGTKLEIK